European Patent Specification EP 3 765 629 B1, published December 25, 2024. Title: KINASE AND/OR PHOSPHATASE SENSING VIA HYDROXYQUINOLINE-SENSITIZED CHELATE. Applicant: Massachusetts Institute of Technology Centre National de la Recherche Scientifique ENSCM UNIVERSITE DE MONTPELLIER. Application Not Yet Assigned. The sequence listing filed with the application follows.

SEQUENCE LISTING (7 sequences)

SEQ ID NO: 1 - protein, 11 aa, Artificial Sequence
  Synthetic polypeptide
LVEPLTPCGEA

SEQ ID NO: 2 - protein, 11 aa, Artificial Sequence
  Synthetic polypeptide
  misc_feature (8)..(8): may be modified by the structure on page 5
LVEPLTPCGEA

SEQ ID NO: 3 - protein, 11 aa, Artificial Sequence
  Synthetic polypeptide
  MOD_RES (6)..(6): PHOSPHORYLATED
  misc_feature (8)..(8): may be modified by the structure on page 5
LVEPLTPCGEA

SEQ ID NO: 4 - protein, 9 aa, Artificial Sequence
  Synthetic polypeptide
  misc_feature (1)..(1): may be modified by an acetyl group
  misc_feature (7)..(7): may be modified by the structure on page 5
EEPIYVCFG

SEQ ID NO: 5 - protein, 5 aa, Artificial Sequence
  Synthetic polypeptide
  misc_feature (3)..(3): may be modified by the structure on page 6
TVCAL

SEQ ID NO: 6 - protein, 5 aa, Artificial Sequence
  Synthetic polypeptide
  misc_feature (3)..(3): may be modified by the structure on page 6
YRCPS

SEQ ID NO: 7 - protein, 4 aa, Artificial Sequence
  Synthetic polypeptide
  misc_feature (1)..(1): may be modified by the structure on page 6
  misc_feature (1)..(1): may be modified by an acetyl group
CGTF